European Patent Application EP 4 711 383 A2, published March 18, 2026. Title: FELINE ANTIBODY VARIANTS. Applicant: Zoetis Services LLC. Application EP. The sequence listing filed with the application follows.

SEQUENCE LISTING (138 sequences)

SEQ ID NO: 1 - protein, 335 aa, Felis catus
ASTTAPSVFPLAPSCGTTSGATVALACLVLGYFPEPVTVSWNSGALTSGVHTFPAVLQASGLYSLSSMVTVPSSRWLSDTFTCNVAHPPSNTKVDKTVRKTDHPPGPKPCDCPKCPPPEMLGGPSIFIFPPKPKDTLSISRTPEVTCLVVDLGPDDSDVQITWFVDNTQVYTAKTSPREEQFNSTYRVVSVLPILHQDWLKGKEFKCKVNSKSLPSPIERTISKAKGQPHEPQVYVLPPAQEELSRNKVSVTCLIKSFHPPDIAVEWEITGQPEPENNYRTTPPQLDSDGTYFVYSKLSVDRSHWQRGNTYTCSVLHEALHSHHTQKSLTQSPGK

SEQ ID NO: 2 - protein, 335 aa, Felis catus
ASTTAPSVFPLAPSCGTTSGATVALACLVLGYFPEPVTVSWNSGALTSGVHTFPAVLQASGLYSLSSMVTVPSSRWLSDTFTCNVAHPPSNTKVDKTVRKTDHPPGPKPCDCPKCPPPEMLGGPSIFIFPPKPKDTLSISRTPEVTCLVVDLGPDDSDVQITWFVDNTQVYTAKTSPREEQFNSTYRVVSVLPILHQDWLKGKEFKCKVNSKSLPSPIERTISKAKGQPHEPQVYVLPPAQEELSRNKVSVTCLIKSFHPPDIAVEWEITGQPEPENNYRTTPPQLDSDGTYFVYSKLSVDRSHWQRGNTYTCSVSHEALHHHHTQKSLTQSPGK

SEQ ID NO: 3 - protein, 335 aa, Felis catus
ASTTAPSVFPLAPSCGTTSGATVALACLVLGYFPEPVTVSWNSGALTSGVHTFPAVLQASGLYSLSSMVTVPSSRWLSDTFTCNVAHPPSNTKVDKTVRKTDHPPGPKPCDCPKCPPPEMLGGPSIFIFPPKPKDTLSISRTPEVTCLVVDLGPDDSDVQITWFVDNTQVYTAKTSPREEQFNSTYRVVSVLPILHQDWLKGKEFKCKVNSKSLPSPIERTISKAKGQPHEPQVYVLPPAQEELSRNKVSVTCLIKSFHPPDIAVEWEITGQPEPENNYRTTPPQLDSDGTYFVYSKLSVDRSHWQRGNTYTCSVSHEALHSHHTQKSLTQSPGK

SEQ ID NO: 4 - DNA, 1005 bp, Felis catus
  source 1..1005: mol_type = genomic DNA
gcctccaccacggccccatcggtgttcccactggcccccagctgcgggaccacatctggcgccaccgtggccctggcctgcctggtgttaggctacttccctgagccggtgaccgtgtcctggaactccggcgccctgaccagcggtgtgcacaccttcccggccgtcctgcaggcctcggggctgtactctctcagcagcatggtgacagtgccctccagcaggtggctcagtgacaccttcacctgcaacgtggcccacccgcccagcaacaccaaggtggacaagaccgtgcgcaaaacagaccacccaccgggacccaaaccctgcgactgtcccaaatgcccaccccctgagatgcttggaggaccgtccatcttcatcttccccccaaaacccaaggacaccctctcgatttcccggacgcccgaggtcacatgcttggtggtggacttgggcccagatgactccgatgtccagatcacatggtttgtggataacacccaggtgtacacagccaagacgagtccgcgtgaggagcagttcaacagcacctaccgtgtggtcagtgtcctccccatcctacaccaggactggctcaaggggaaggagttcaagtgcaaggtcaacagcaaatccctcccctcccccatcgagaggaccatctccaaggccaaaggacagccccacgagccccaggtgtacgtcctgcctccagcccaggaggagctcagcaggaacaaagtcagtgtgacctgcctgatcaaatccttccacccgcctgacattgccgtcgagtgggagatcaccggacagccggagccagagaacaactaccggacgaccccgccccagctggacagcgacgggacctacttcgtgtacagcaagctctcggtggacaggtcccactggcagaggggaaacacctacacctgctcggtgtcacacgaagctctgcacagccaccacacacagaaatccctcacccagtctccgggtaaa

SEQ ID NO: 5 - protein, 98 aa, Felis catus
ASTTAPSVFPLAPSCGTTSGATVALACLVLGYFPEPVTVSWNSGALTSGVHTFPAVLQASGLYSLSSMVTVPSSRWLSDTFTCNVAHPPSNTKVDKTV

SEQ ID NO: 6 - protein, 18 aa, Felis catus
RKTDHPPGPKPCDCPKCP

SEQ ID NO: 7 - protein, 110 aa, Felis catus
PPEMLGGPSIFIFPPKPKDTLSISRTPEVTCLVVDLGPDDSDVQITWFVDNTQVYTAKTSPREEQFNSTYRVVSVLPILHQDWLKGKEFKCKVNSKSLPSPIERTISKAK

SEQ ID NO: 8 - protein, 109 aa, Felis catus
GQPHEPQVYVLPPAQEELSRNKVSVTCLIKSFHPPDIAVEWEITGQPEPENNYRTTPPQLDSDGTYFVYSKLSVDRSHWQRGNTYTCSVSHEALHSHHTQKSLTQSPGK

SEQ ID NO: 9 - DNA, 294 bp, Felis catus
  source 1..294: mol_type = genomic DNA
gcctccaccacggccccatcggtgttcccactggcccccagctgcgggaccacatctggcgccaccgtggccctggcctgcctggtgttaggctacttccctgagccggtgaccgtgtcctggaactccggcgccctgaccagcggtgtgcacaccttcccggccgtcctgcaggcctcggggctgtactctctcagcagcatggtgacagtgccctccagcaggtggctcagtgacaccttcacctgcaacgtggcccacccgcccagcaacaccaaggtggacaagaccgtg

SEQ ID NO: 10 - DNA, 54 bp, Felis catus
  source 1..54: mol_type = genomic DNA
cgcaaaacagaccacccaccgggacccaaaccctgcgactgtcccaaatgccca

SEQ ID NO: 11 - DNA, 330 bp, Felis catus
  source 1..330: mol_type = genomic DNA
ccccctgagatgcttggaggaccgtccatcttcatcttccccccaaaacccaaggacaccctctcgatttcccggacgcccgaggtcacatgcttggtggtggacttgggcccagatgactccgatgtccagatcacatggtttgtggataacacccaggtgtacacagccaagacgagtccgcgtgaggagcagttcaacagcacctaccgtgtggtcagtgtcctccccatcctacaccaggactggctcaaggggaaggagttcaagtgcaaggtcaacagcaaatccctcccctcccccatcgagaggaccatctccaaggccaaa

SEQ ID NO: 12 - DNA, 327 bp, Felis catus
  source 1..327: mol_type = genomic DNA
ggacagccccacgagccccaggtgtacgtcctgcctccagcccaggaggagctcagcaggaacaaagtcagtgtgacctgcctgatcaaatccttccacccgcctgacattgccgtcgagtgggagatcaccggacagccggagccagagaacaactaccggacgaccccgccccagctggacagcgacgggacctacttcgtgtacagcaagctctcggtggacaggtcccactggcagaggggaaacacctacacctgctcggtgtcacacgaagctctgcacagccaccacacacagaaatccctcacccagtctccgggtaaa

SEQ ID NO: 13 - DNA, 351 bp, synthetic construct
  misc_feature 1..351: note = ZTS-5864 Heavy Chain Variable Region
  source 1..351: mol_type = other DNA
gacgtgcaattggtggagtctgggggagacctggtgaagcctggggggtccctgagactcacctgtgtggcctctggattcaccttcagtgactatgcaatgagctgggtccgccaggctccagggaaggggctgcagtgggtcgcaggtattgacagtgttggaagtggcacaagctacgcagactccgtgaagggccgattcaccatctccagagacaatgccaagaacacgctgtatctgcagatgaacagcctcaagaccgaggacacggccacatattactgtgcgagcgggttccctgggtcctttgagcactggggccaaggaaccctggtgacggtctcgagc

SEQ ID NO: 14 - protein, 117 aa, synthetic construct
  REGION 1..117: note = ZTS-5864 Heavy Chain Variable Region
DVQLVESGGDLVKPGGSLRLTCVASGFTFSDYAMSWVRQAPGKGLQWVAGIDSVGSGTSYADSVKGRFTISRDNAKNTLYLQMNSLKTEDTATYYCASGFPGSFEHWGQGTLVTVSS

SEQ ID NO: 15 - protein, 5 aa, Canis familiaris
DYAMS

SEQ ID NO: 16 - protein, 17 aa, Canis familiaris
GIDSVGSGTSYADSVKG

SEQ ID NO: 17 - protein, 8 aa, Canis familiaris
GFPGSFEH

SEQ ID NO: 18 - DNA, 312 bp, synthetic construct
  misc_feature 1..312: note = ZTS-5864 Light Chain Variable Region
  source 1..312: mol_type = other DNA
cagtctgtgctgactcagccatcctcagtgtctgggaccctaggccagaggatcaccatctcctgcaccggaagcagctccaacatcgggagtggttatgtgggctggtatcaacaagtcccaggaatgggccccaaaaccgtcatctattataatagcgaccgaccctctggagtcccagataggttctccggctccaagtctggcagctcaggcaccctgaccatcactggattgcaggctgaagacgaggctgactattactgttcagtatatgacagaactttcaatgctgtgttcggcggagggacc

SEQ ID NO: 19 - protein, 104 aa, synthetic construct
  REGION 1..104: note = ZTS-5864 Light Chain Variable Region
QSVLTQPSSVSGTLGQRITISCTGSSSNIGSGYVGWYQQVPGMGPKTVIYYNSDRPSGVPDRFSGSKSGSSGTLTITGLQAEDEADYYCSVYDRTFNAVFGGGT

SEQ ID NO: 20 - protein, 13 aa, Canis familiaris
TGSSSNIGSGYVG

SEQ ID NO: 21 - protein, 7 aa, Canis familiaris
YYNSDRP

SEQ ID NO: 22 - protein, 10 aa, Canis familiaris
SVYDRTFNAV

SEQ ID NO: 23 - protein, 453 aa, synthetic construct
  REGION 1..453: note = ZTS768_Heavy_chain
DVQLVESGGDLVKPGGSLRLTCVASGFTYSNYWMHWVRQAPGKGLQWVARIDPYGGGTKHNEKFKRRFTISRDNAKNTLYLQMNSLKTEDTATYYCVRSGYDYYFDVWGQGTLVTVSSASTTAPSVFPLAPSCGTTSGATVALACLVLGYFPEPVTVSWNSGALTSGVHTFPAVLQASGLYSLSSMVTVPSSRWLSDTFTCNVAHPPSNTKVDKTVRKTDHPPGPKPCDCPKCPPPEMLGGPSIFIFPPKPKDTLSISRTPEVTCLVVDLGPDDSDVQITWFVDNTQVYTAKTSPREEQFNSTYRVVSVLPILHQDWLKGKEFKCKVNSKSLPSPIERTISKAKGQPHEPQVYVLPPAQEELSRNKVSVTCLIKSFHPPDIAVEWEITGQPEPENNYRTTPPQLDSDGTYFVYSKLSVDRSHWQRGNTYTCSVSHEALHSHHTQKSLTQSPGK

SEQ ID NO: 24 - protein, 5 aa, Mus musculus
NYWMH

SEQ ID NO: 25 - protein, 17 aa, Mus musculus
RIDPYGGGTKHNEKFKR

SEQ ID NO: 26 - protein, 9 aa, Mus musculus
SGYDYYFDV

SEQ ID NO: 27 - protein, 217 aa, synthetic construct
  REGION 1..217: note = ZTS768_Light_chain
EIQMTQSPSSLSASPGDRVTITCRASENIYSFLAWYQQKPGKVPKLLIYNANTLAEGVPSRFSGSGSGTDFTLTISSLEPEDAATYYCQHHFGTPFTFGSGTKLEIKRSDAQPSVFLFQPSLDELHTGSASIVCILNDFYPKEVNVKWKVDGVVQNKGIQESTTEQNSKDSTYSLSSTLTMSSTEYQSHEKFSCEVTHKSLASTLVKSFQRSECQRE

SEQ ID NO: 28 - protein, 11 aa, Mus musculus
RASENIYSFLA

SEQ ID NO: 29 - protein, 7 aa, Mus musculus
NANTLAE

SEQ ID NO: 30 - protein, 9 aa, Mus musculus
QHHFGTPFT

SEQ ID NO: 31 - protein, 457 aa, synthetic construct
  REGION 1..457: note = NV02_Heavy chain
QVQLVESGAELVQPGESLRLTCAASGFSLTNNNVNWVRQAPGKGLEWMGGVWAGGATDYNSALKSRLTITRDTSKNTVFLQMHSLQSEDTATYYCARDGGYSSSTLYAMDAWGQGTTVTVSAASTTAPSVFPLAPSCGTTSGATVALACLVLGYFPEPVTVSWNSGALTSGVHTFPAVLQASGLYSLSSMVTVPSSRWLSDTFTCNVAHPPSNTKVDKTVRKTDHPPGPKPCDCPKCPPPEMLGGPSIFIFPPKPKDTLSISRTPEVTCLVVDLGPDDSDVQITWFVDNTQVYTAKTSPREEQFNSTYRVVSVLPILHQDWLKGKEFKCKVNSKSLPSPIERTISKAKGQPHEPQVYVLPPAQEELSRNKVSVTCLIKSFHPPDIAVEWEITGQPEPENNYRTTPPQLDSDGTYFVYSKLSVDRSHWQRGNTYTCSVSHEALHSHHTQKSLTQSPGK

SEQ ID NO: 32 - protein, 10 aa, Rattus rattus
GFSLTNNNVN

SEQ ID NO: 33 - protein, 16 aa, Rattus rattus
GVWAGGATDYNSALKS

SEQ ID NO: 34 - protein, 14 aa, Rattus rattus
DGGYSSSTLYAMDA

SEQ ID NO: 35 - protein, 217 aa, synthetic construct
  REGION 1..217: note = >NV02_Kappa chain
DIEMTQSPLSLSVTPGESVSISCRASEDIYNALAWYLQKPGRSPRLLIYNTDTLHTGVPDRFSGSGSGTDFTLKISRVQTEDVGVYFCQHYFHYPRTFGQGTKLELKRSDAQPSVFLFQPSLDELHTGSASIVCILNDFYPKEVNVKWKVDGVVQNKGIQESTTEQNSKDSTYSLSSTLTMSSTEYQSHEKFSCEVTHKSLASTLVKSFQRSECQRE

SEQ ID NO: 36 - protein, 11 aa, Rattus rattus
RASEDIYNALA

SEQ ID NO: 37 - protein, 7 aa, Rattus rattus
NTDTLHT

SEQ ID NO: 38 - protein, 9 aa, Rattus rattus
QHYFHYPRT

SEQ ID NO: 39 - protein, 5 aa, Mus musculus
SSWMN

SEQ ID NO: 40 - protein, 17 aa, Mus musculus
QIYPGDGDTNYNGKFKG

SEQ ID NO: 41 - protein, 10 aa, Mus musculus
ARHYDGSTDY

SEQ ID NO: 42 - protein, 11 aa, Mus musculus
RASENIYSNLA

SEQ ID NO: 43 - protein, 7 aa, Mus musculus
AATNLAD

SEQ ID NO: 44 - protein, 9 aa, Mus musculus
QHFWGTPYT

SEQ ID NO: 45 - protein, 117 aa, synthetic construct
  REGION 1..117: note = Felinized Sequence - Variable Heavy Region Engineered to Have Sequences from Mus musculus and Felis
QVLLVQSGAEVRRPGASVKIFCKASGYSFTSSWMNWLRQAPAQGFEWMGQIYPGDGDTNYNGKFKGRLTLTADTSTDTAYMELSSLRSADTAVYYCARHYDGSTDYWGHGTIVTVSS

SEQ ID NO: 46 - DNA, 351 bp, synthetic construct
  misc_feature 1..351: note = Felinized Sequence - Variable Heavy Region Engineered to Have Sequences from Mus musculus and Felis
  source 1..351: mol_type = other DNA
caggtgctgctggtgcagagcggcgcggaagtgcgccgcccgggcgcgagcgtgaaaattttttgcaaagcgagcggctatagctttaccagcagctggatgaactggctgcgccaggcgccggcgcagggctttgaatggatgggccagatttatccgggcgatggcgataccaactataacggcaaatttaaaggccgcctgaccctgaccgcggataccagcaccgataccgcgtatatggaactgagcagcctgcgcagcgcggataccgcggtgtattattgcgcgcgccattatgatggcagcaccgattattggggccatggcaccattgtgaccgtgagcagc

SEQ ID NO: 47 - protein, 103 aa, synthetic construct
  REGION 1..103: note = Felinized Sequence - Variable Light Region Engineered to Have Sequences from Mus musculus and Felis
AITMTQSPGSLAGSPGQQVTMNCRASENIYSNLAWYQQKPGQHPKLLIYAATNLADGVPDRFSGSGSGTDFTLTISNLQAEDVASYYCQHFWGTPYTFGGGTK

SEQ ID NO: 48 - DNA, 309 bp, synthetic construct
  misc_feature 1..309: note = Felinized Sequence - Variable Light Region Engineered to Have Sequences from Mus musculus and Felis
  source 1..309: mol_type = other DNA
gcgattaccatgacccagagcccgggcagcctggcgggcagcccgggccagcaggtgaccatgaactgccgcgcgagcgaaaacatttatagcaacctggcgtggtatcagcagaaaccgggccagcatccgaaactgctgatttatgcggcgaccaacctggcggatggcgtgccggatcgctttagcggcagcggcagcggcaccgattttaccctgaccattagcaacctgcaggcggaagatgtggcgagctattattgccagcatttttggggcaccccgtatacctttggcggcggcaccaaa

SEQ ID NO: 49 - protein, 5 aa, Homo sapiens
SNVIS

SEQ ID NO: 50 - protein, 18 aa, Homo sapiens
GVIPIVDIANYAQRFKGR

SEQ ID NO: 51 - protein, 11 aa, Homo sapiens
TLGLVLDAMDY

SEQ ID NO: 52 - protein, 10 aa, Homo sapiens
RASQSLGSSY

SEQ ID NO: 53 - protein, 7 aa, Homo sapiens
GASSRAP

SEQ ID NO: 54 - protein, 9 aa, Homo sapiens
QQYADSPIT

SEQ ID NO: 55 - protein, 120 aa, synthetic construct
  REGION 1..120: note = Felinized Sequence - Variable Heavy Region Engineered to Have Sequences from Homo sapiens and Felis
QVQLVQSGAEVKKPGSSVKVSCKASGYTFSSNVISWVRQAPGQGLEWMGGVIPIVDIANYAQRFKGRVTITADESTSTTYMELSSLRSEDTAVYYCASTLGLVLDAMDYWGQGTLVTVSS

SEQ ID NO: 56 - DNA, 360 bp, synthetic construct
  misc_feature 1..360: note = Felinized Sequence - Variable Heavy Region Engineered to Have Sequences from Homo sapiens and Felis
  source 1..360: mol_type = other DNA
caggtgcagctggtgcagtccggagctgaggtgaagaagccaggctccagcgtgaaggtgtcttgcaaggcttccggctacaccttctcttccaacgtgatcagctgggtgagacaggctccaggacagggactggagtggatgggaggcgtgatccctatcgtggacatcgccaattacgctcagaggtttaagggccgggtgaccatcacagctgatgagtccacaagcaccacatatatggagctgagctctctgcgcagcgaggacaccgccgtgtactattgtgcttctacactgggcctggtgctggacgctatggactattggggccagggcaccctggtgacagtctcgagc

SEQ ID NO: 57 - protein, 108 aa, synthetic construct
  REGION 1..108: note = Felinized Sequence - Variable Light Region Engineered to Have Sequences from Homo sapiens and Felis
ETVLTQSPGTLSLSPGERATLSCRASQSLGSSYLAWYQQKPGQAPRLLIYGASSRAPGIPDRFSGSGSGTDFTLTISRLEPEDFAVYYCQQYADSPITFGQGTKLEIK

SEQ ID NO: 58 - DNA, 324 bp, synthetic construct
  misc_feature 1..324: note = Felinized Sequence - Variable Light Region Engineered to Have Sequences from Homo sapiens and Felis
  source 1..324: mol_type = other DNA
gagaccgtgctgacacagtctcctggcaccctgagcctgtctccaggagagagggccacactgtcctgcagggcttcccagagcctgggctccagctacctggcctggtatcagcagaagccaggccaggctcccaggctgctgatctacggagcctcttccagagctccaggcatccctgaccgcttctctggatccggaagcggcaccgacttcaccctgacaatcagcagactggagcccgaggacttcgccgtgtactattgtcagcagtatgctgattctcctatcacatttggccagggtaccaagctggagatcaaa

SEQ ID NO: 59 - protein, 5 aa, Homo sapiens
SNVIS

SEQ ID NO: 60 - protein, 17 aa, Homo sapiens
GVIPIVDIANYAQRFKG

SEQ ID NO: 61 - protein, 13 aa, Homo sapiens
ASTLGLVLDAMDY

SEQ ID NO: 62 - protein, 10 aa, Homo sapiens
RASQSLGSSY

SEQ ID NO: 63 - protein, 7 aa, Homo sapiens
GASSRAP

SEQ ID NO: 64 - protein, 9 aa, Homo sapiens
QQYADSPIT

SEQ ID NO: 65 - protein, 120 aa, synthetic construct
  REGION 1..120: note = Felinized Sequence - Variable Heavy Region Engineered to Have Sequences from Homo sapiens and Felis
QVLLVQSGADVRKPGASVKIFCKASGYTFTSNVISWVRQTPAQGFEWMGGVIPIVDIANYAQRFKGRLVLTADTSTNTAYMELRSLKSADTAVYYCASTLGLVLDAMDYWGQGSLVTVSS

SEQ ID NO: 66 - DNA, 360 bp, synthetic construct
  misc_feature 1..360: note = Felinized Sequence - Variable Heavy Region Engineered to Have Sequences from Homo sapiens and Felis
  source 1..360: mol_type = other DNA
caggtgctgctggtgcagtctggcgccgatgtgagaaagccaggcgctagcgtgaagatcttctgcaaggcctctggctacacctttacatctaacgtgatctcctgggtgcgccagacaccagctcagggattcgagtggatgggaggcgtgatccctatcgtggacatcgccaactacgctcagaggtttaagggccggctggtgctgaccgctgatacctccacaaataccgcttatatggagctgaggtccctgaagagcgccgacacagccgtgtactattgtgcctccaccctgggactggtgctggacgctatggattattggggccagggcagcctggtgacagtctcgagc

SEQ ID NO: 67 - protein, 108 aa, synthetic construct
  REGION 1..108: note = Felinized Sequence - Variable Light Region Engineered to Have Sequences from Homo sapiens and Felis
EIQMTQSPSSLSASPGDRVTITCRASQSLGSSYLAWYQQKPGKVPKLLIYGASSRAPGVPSRFSGSGSGTDFTLTISSLEPEDAATYYCQQYADSPITFGQGTKLEIK

SEQ ID NO: 68 - DNA, 324 bp, synthetic construct
  misc_feature 1..324: note = Felinized Sequence - Variable Light Region Engineered to Have Sequences from Homo sapiens and Felis
  source 1..324: mol_type = other DNA
gagatccagatgacccagtctccttccagcctgtctgcctccccaggcgacagggtgaccatcacatgccgggccagccagtctctgggctcttcctacctggcttggtatcagcagaagccaggcaaggtgcccaagctgctgatctacggagccagctctagagctccaggcgtgccttcccgcttctccggaagcggatctggcacagacttcaccctgacaatctccagcctggagccagaggacgctgctacctactattgtcagcagtatgctgatagccctatcacattcggccagggtaccaagctggagatcaaa

SEQ ID NO: 69 - protein, 5 aa, Homo sapiens
SNVIS

SEQ ID NO: 70 - protein, 17 aa, Homo sapiens
GVIPIVDIANYAQRFKG

SEQ ID NO: 71 - protein, 13 aa, Homo sapiens
ASTLGLVLDAMDY

SEQ ID NO: 72 - protein, 12 aa, Homo sapiens
RASQSLGSSYLA

SEQ ID NO: 73 - protein, 7 aa, Homo sapiens
GASSRAP

SEQ ID NO: 74 - protein, 9 aa, Homo sapiens
QQYADSPIT

SEQ ID NO: 75 - protein, 120 aa, synthetic construct
  REGION 1..120: note = Felinized Sequence - Variable Heavy Region Engineered to Have Sequences from Homo sapiens and Felis
QVLLVQSGAEVRTPGASVKIFCKASGYGFTSNVISWVRQSPAQGLEWMGGVIPIVDIANYAQRFKGRLTLTADTSTDTAYMELSSLRSADTAMYYCASTLGLVLDAMDYWGQGTLVTVSS

SEQ ID NO: 76 - DNA, 363 bp, synthetic construct
  misc_feature 1..363: note = Felinized Sequence - Variable Heavy Region Engineered to Have Sequences from Homo sapiens and Felis
  source 1..363: mol_type = other DNA
caggtgctgctggtgcagtctggcgccgaggtgagaacaccaggcgctagcgtgaagatcttctgcaaggcctctggctacggctttacctctaacgtgatctcctgggtgcgccagtccccagctcagggactggagtggatgggaggcgtgatccctatcgtggacatcgccaattacgctcagaggttcaagggccggctgaccctgacagctgacacctccacagataccgcttatatggagctgtccagcctgaggtccgccgatacagctatgtactattgtgccagcaccctgggactggtgctggacgctatggattattggggccagggcacactggtgaccgtggtctcgagc

SEQ ID NO: 77 - protein, 108 aa, synthetic construct; identical to SEQ ID NO: 67
  REGION 1..108: note = Felinized Sequence - Variable Light Region Engineered to Have Sequences from Homo sapiens and Felis

SEQ ID NO: 78 - DNA, 324 bp, synthetic construct; identical to SEQ ID NO: 68
  misc_feature 1..324: note = Felinized Sequence - Variable Light Region Engineered to Have Sequences from Homo sapiens and Felis
  source 1..324: mol_type = other DNA

SEQ ID NO: 79 - protein, 8 aa, Homo sapiens
GYTFSSNV

SEQ ID NO: 80 - protein, 8 aa, Homo sapiens
VIPIVDIA

SEQ ID NO: 81 - protein, 10 aa, Homo sapiens
LGLVLDAMDY

SEQ ID NO: 82 - protein, 12 aa, Homo sapiens
RASQSLGSSYLA

SEQ ID NO: 83 - protein, 7 aa, Homo sapiens
GASSRAP

SEQ ID NO: 84 - protein, 9 aa, Homo sapiens
QQYADSPIT

SEQ ID NO: 85 - protein, 120 aa, synthetic construct
  REGION 1..120: note = Felinized Sequence - Variable Heavy Region Engineered to Have Sequences from Homo sapiens and Felis
QVLLVQSGADVRKPGASVKIFCKASGYTFSSNVMHWVRQTPAQGFEWMGSVIPIVDIATYARRFQGRLVLTADTSTNTAYMELRSLKSADTAVYYCARTLGLVLDAMDYWGQGSLVTVSS

SEQ ID NO: 86 - DNA, 360 bp, synthetic construct
  misc_feature 1..360: note = Felinized Sequence - Variable Heavy Region Engineered to Have Sequences from Homo sapiens and Felis
  source 1..360: mol_type = other DNA
caggtgctgctggtgcagtctggcgccgatgtgaggaagccaggcgctagcgtgaagatcttctgcaaggcctctggctacacattttccagcaacgtgatgcactgggtgagacagacccccgctcagggcttcgagtggatgggctccgtgatccctatcgtggacatcgccacatacgctaggcggtttcagggcaggctggtgctgaccgccgataccagcacaaataccgcttatatggagctgagatctctgaagtccgccgacacagccgtgtactattgtgctcgcaccctgggactggtgctggacgctatggattattggggccagggctccctggtgacagtctcgagc

SEQ ID NO: 87 - protein, 108 aa, synthetic construct; identical to SEQ ID NO: 67
  REGION 1..108: note = Felinized Sequence - Variable Light Region Engineered to Have Sequences from Homo sapiens and Felis

SEQ ID NO: 88 - DNA, 324 bp, synthetic construct; identical to SEQ ID NO: 68
  misc_feature 1..324: note = Felinized Sequence - Variable Light Region Engineered to Have Sequences from Homo sapiens and Felis
  source 1..324: mol_type = other DNA

SEQ ID NO: 89 - protein, 8 aa, Homo sapiens
GYTFSSNV

SEQ ID NO: 90 - protein, 8 aa, Homo sapiens
VIPIVDIA

SEQ ID NO: 91 - protein, 8 aa, Homo sapiens
LVLDAMDY

SEQ ID NO: 92 - protein, 12 aa, Homo sapiens
RASQSLGSSYLA

SEQ ID NO: 93 - protein, 7 aa, Homo sapiens
GASSRAP

SEQ ID NO: 94 - protein, 9 aa, Homo sapiens
QQYADSPIT

SEQ ID NO: 95 - protein, 120 aa, synthetic construct
  REGION 1..120: note = Felinized Sequence - Variable Heavy Region Engineered to Have Sequences from Homo sapiens and Felis
DVQLVESGGDLVKPGGSLRLTCVASGYTFSSNVMHWVRQAPGKGLQWVAYVIPIVDIAYYADSVKGRFTISIDNSKNTLYLQMNSLKTEDTATYYCARTLGLVLDAMDYWGQGTLVTVSS

SEQ ID NO: 96 - DNA, 360 bp, synthetic construct
  misc_feature 1..360: note = Felinized Sequence - Variable Heavy Region Engineered to Have Sequences from Homo sapiens and Felis
  source 1..360: mol_type = other DNA
gacgtgcagctggtggagtctggaggcgatctggtgaagccaggaggcagcctgaggctgacctgcgtggcttctggctacacattctccagcaacgtgatgcactgggtgcggcaggctccaggcaagggactgcagtgggtggcttatgtgatccctatcgtggacatcgcctactatgctgattccgtgaagggcaggttcaccatctctatcgacaactccaagaatacactgtacctgcagatgaatagcctgaagaccgaggataccgccacatactattgtgctcgcacactgggcctggtgctggacgctatggattattggggccagggcaccctggtgacagtctcgagc

SEQ ID NO: 97 - protein, 108 aa, synthetic construct; identical to SEQ ID NO: 67
  REGION 1..108: note = Felinized Sequence - Variable Light Region Engineered to Have Sequences from Homo sapiens and Felis

SEQ ID NO: 98 - DNA, 324 bp, synthetic construct; identical to SEQ ID NO: 68
  misc_feature 1..324: note = Felinized Sequence - Variable Light Region Engineered to Have Sequences from Homo sapiens and Felis
  source 1..324: mol_type = other DNA

SEQ ID NO: 99 - protein, 8 aa, Homo sapiens
GYTFSSNV

SEQ ID NO: 100 - protein, 8 aa, Homo sapiens
VIPIVDIA

SEQ ID NO: 101 - protein, 10 aa, Homo sapiens
LGLVLDAMDY

SEQ ID NO: 102 - protein, 12 aa, Homo sapiens
RASQSLGSSYLA

SEQ ID NO: 103 - protein, 7 aa, Homo sapiens
GASSRAP

SEQ ID NO: 104 - protein, 9 aa, Homo sapiens
QQYADSPIT

SEQ ID NO: 105 - protein, 120 aa, synthetic construct; identical to SEQ ID NO: 85
  REGION 1..120: note = Felinized Sequence - Variable Heavy Region Engineered to Have Sequences from Homo sapiens and Felis

SEQ ID NO: 106 - DNA, 360 bp, synthetic construct; identical to SEQ ID NO: 86
  misc_feature 1..360: note = Felinized Sequence - Variable Heavy Region Engineered to Have Sequences from Homo sapiens and Felis
  source 1..360: mol_type = other DNA

SEQ ID NO: 107 - protein, 107 aa, synthetic construct
  REGION 1..107: note = Felinized Sequence - Variable Light Region Engineered to Have Sequences from Homo sapiens and Felis
DIVLTQPPSLSVNLGQTARITCRASQSLGSSYLAWYQQKPGQAPKLVTYGASSRAPGIPDRFSGTNSGITATLTISGARAEDEADYYCQQYADSPITFGQGTKLEIK

SEQ ID NO: 108 - DNA, 321 bp, synthetic construct
  misc_feature 1..321: note = Felinized Sequence - Variable Light Region Engineered to Have Sequences from Homo sapiens and Felis
  source 1..321: mol_type = other DNA
gacatcgtgctgacacagccccctagcctgtctgtgaacctgggacagacagctaggatcacctgcagggcttcccagagcctgggctccagctacctggcctggtatcagcagaagcctggccaggctccaaagctggtgacatacggcgcctcttccagagctccaggcatccccgaccgcttctctggcaccaattccggcatcaccgccacactgaccatcagcggagccagggctgaggacgaggctgattactattgtcagcagtatgctgattctcccatcacctttggccagggtaccaagctggagatcaaa

SEQ ID NO: 109 - protein, 8 aa, Homo sapiens
GYTFSSNV

SEQ ID NO: 110 - protein, 8 aa, Homo sapiens
VIPIVDIA

SEQ ID NO: 111 - protein, 8 aa, Homo sapiens
LVLDAMDY

SEQ ID NO: 112 - protein, 12 aa, Homo sapiens
RASQSLGSSYLA

SEQ ID NO: 113 - protein, 7 aa, Homo sapiens
GASSRAP

SEQ ID NO: 114 - protein, 9 aa, Homo sapiens
QQYADSPIT

SEQ ID NO: 115 - protein, 120 aa, synthetic construct; identical to SEQ ID NO: 95
  REGION 1..120: note = Felinized Sequence - Variable Heavy Region Engineered to Have Sequences from Homo sapiens and Felis

SEQ ID NO: 116 - DNA, 360 bp, synthetic construct; identical to SEQ ID NO: 96
  misc_feature 1..360: note = Felinized Sequence - Variable Heavy Region Engineered to Have Sequences from Homo sapiens and Felis
  source 1..360: mol_type = other DNA

SEQ ID NO: 117 - protein, 107 aa, synthetic construct; identical to SEQ ID NO: 107
  REGION 1..107: note = Felinized Sequence - Variable Light Region Engineered to Have Sequences from Homo sapiens and Felis

SEQ ID NO: 118 - DNA, 321 bp, synthetic construct; identical to SEQ ID NO: 108
  misc_feature 1..321: note = Felinized Sequence - Variable Light Region Engineered to Have Sequences from Homo sapiens and Felis
  source 1..321: mol_type = other DNA

SEQ ID NO: 119 - protein, 5 aa, Homo sapiens
SNVIS

SEQ ID NO: 120 - protein, 17 aa, Homo sapiens
GVIPIVDIANYAQRFKG

SEQ ID NO: 121 - protein, 13 aa, Homo sapiens
ASTLGLVLDAMDY

SEQ ID NO: 122 - protein, 12 aa, Homo sapiens
RASQSLGSSYLA

SEQ ID NO: 123 - protein, 7 aa, Homo sapiens
GASSRAP

SEQ ID NO: 124 - protein, 9 aa, Homo sapiens
QQYADSPIT

SEQ ID NO: 125 - protein, 120 aa, synthetic construct; identical to SEQ ID NO: 65
  REGION 1..120: note = Felinized Sequence - Variable Heavy Region Engineered to Have Sequences from Homo sapiens and Felis

SEQ ID NO: 126 - DNA, 360 bp, synthetic construct; identical to SEQ ID NO: 66
  misc_feature 1..360: note = Felinized Sequence - Variable Heavy Region Engineered to Have Sequences from Homo sapiens and Felis
  source 1..360: mol_type = other DNA

SEQ ID NO: 127 - protein, 108 aa, synthetic construct
  REGION 1..108: note = Felinized Sequence - Variable Light Region Engineered to Have Sequences from Homo sapiens and Felis
DIVMTQSPGSLAGSPGQQVTMNCRASQSLGSSYLAWYQQKPGQHPELLIYGASSRAPGVPDRFSGSGSGTDFTLTISNLQAEDVANYYCQQYADSPITFGQGTKLEIK

SEQ ID NO: 128 - DNA, 324 bp, synthetic construct
  misc_feature 1..324: note = Felinized Sequence - Variable Light Region Engineered to Have Sequences from Homo sapiens and Felis
  source 1..324: mol_type = other DNA
gacatcgtgatgacccagtcccctggcagcctggctggaagcccaggacagcaggtgacaatgaactgcagggccagccagtctctgggctccagctacctggcttggtatcagcagaagccaggccagcaccccgagctgctgatctacggagcctcttccagggctccaggcgtgcctgaccggttctccggaagcggatctggcaccgacttcaccctgacaatctctaacctgcaggccgaggacgtggctaattactattgtcagcagtatgctgattcccccatcacattcggccagggtaccaagctggagatcaaa

SEQ ID NO: 129 - protein, 8 aa, Homo sapiens
GYTFSSNV

SEQ ID NO: 130 - protein, 8 aa, Homo sapiens
VIPIVDIA

SEQ ID NO: 131 - protein, 8 aa, Homo sapiens
LVLDAMDY

SEQ ID NO: 132 - protein, 12 aa, Homo sapiens
RASQSLGSSYLA

SEQ ID NO: 133 - protein, 7 aa, Homo sapiens
GASSRAP

SEQ ID NO: 134 - protein, 9 aa, Homo sapiens
QQYADSPIT

SEQ ID NO: 135 - protein, 120 aa, synthetic construct; identical to SEQ ID NO: 95
  REGION 1..120: note = Felinized Sequence - Variable Heavy Region Engineered to Have Sequences from Homo sapiens and Felis

SEQ ID NO: 136 - DNA, 360 bp, synthetic construct; identical to SEQ ID NO: 96
  misc_feature 1..360: note = Felinized Sequence - Variable Heavy Region Engineered to Have Sequences from Homo sapiens and Felis
  source 1..360: mol_type = other DNA

SEQ ID NO: 137 - protein, 108 aa, synthetic construct; identical to SEQ ID NO: 127
  REGION 1..108: note = Felinized Sequence - Variable Light Region Engineered to Have Sequences from Homo sapiens and Felis

SEQ ID NO: 138 - DNA, 324 bp, synthetic construct; identical to SEQ ID NO: 128
  misc_feature 1..324: note = Felinized Sequence - Variable Light Region Engineered to Have Sequences from Homo sapiens and Felis
  source 1..324: mol_type = other DNA